European Patent Application EP 4 273 244 A1, published November 8, 2023. Title: Nucleic acid fragment and use thereof. Applicant: Kyushu University. The sequence listing filed with the application follows.

SEQUENCE LISTING (11 sequences)

SEQ ID NO: 1 - DNA, 70 bp, Artificial Sequence
  Synthesized oligonucleotide
  misc_feature (1)..(1): Azide-modified nucleotide
cccatgcattaatacgactcactatagggtagatcgctcgtcggcagcgtcagatgtgtataagagacag

SEQ ID NO: 2 - DNA, 70 bp, Artificial Sequence
  Synthesized oligonucleotide
  misc_feature (1)..(1): Phosphate-modified nucleotide
  misc_feature (70)..(70): TAMRA-modified nucleotide
ctgtctcttatacacatctgacgctgccgacgagcgatctaccctatagtgagtcgtattaatgcatggg

SEQ ID NO: 3 - DNA, 70 bp, Artificial Sequence; identical to SEQ ID NO: 2
  Synthesized oligonucleotide
  misc_feature (1)..(1): Phosphate-modified nucleotide
  misc_feature (45)..(45): NPOM-dTMP
  misc_feature (50)..(50): NPOM-dTMP
  misc_feature (54)..(54): NPOM-dTMP
  misc_feature (57)..(57): NPOM-dTMP
  misc_feature (59)..(59): NPOM-dTMP
  misc_feature (60)..(60): NPOM-dTMP
  misc_feature (70)..(70): TAMRA-modified nucleotide

SEQ ID NO: 4 - DNA, 70 bp, Artificial Sequence; identical to SEQ ID NO: 2
  Synthesized oligonucleotide
  misc_feature (1)..(1): Phosphate-modified nucleotide
  misc_feature (45)..(45): NPOM-dTMP
  misc_feature (50)..(50): NPOM-dTMP
  misc_feature (54)..(54): NPOM-dTMP
  misc_feature (57)..(57): NPOM-dTMP
  misc_feature (70)..(70): TAMRA-modified nucleotide

SEQ ID NO: 5 - DNA, 70 bp, Artificial Sequence; identical to SEQ ID NO: 2
  Synthesized oligonucleotide
  misc_feature (1)..(1): Phosphate-modified nucleotide
  misc_feature (38)..(38): NPOM-dTMP
  misc_feature (40)..(40): NPOM-dTMP
  misc_feature (47)..(47): NPOM-dTMP
  misc_feature (50)..(50): NPOM-dTMP
  misc_feature (54)..(54): NPOM-dTMP
  misc_feature (57)..(57): NPOM-dTMP
  misc_feature (70)..(70): TAMRA-modified nucleotide

SEQ ID NO: 6 - DNA, 70 bp, Artificial Sequence; identical to SEQ ID NO: 2
  Synthesized oligonucleotide
  misc_feature (1)..(1): Phosphate-modified nucleotide
  misc_feature (8)..(8): NPOM-dTMP
  misc_feature (9)..(9): NPOM-dTMP
  misc_feature (11)..(11): NPOM-dTMP
  misc_feature (17)..(17): NPOM-dTMP
  misc_feature (19)..(19): NPOM-dTMP
  misc_feature (25)..(25): NPOM-dTMP
  misc_feature (70)..(70): TAMRA-modified nucleotide

SEQ ID NO: 7 - DNA, 70 bp, Artificial Sequence; identical to SEQ ID NO: 2
  Synthesized oligonucleotide
  misc_feature (1)..(1): Phosphate-modified nucleotide
  misc_feature (11)..(11): NPOM-dTMP
  misc_feature (17)..(17): NPOM-dTMP
  misc_feature (19)..(19): NPOM-dTMP
  misc_feature (25)..(25): NPOM-dTMP
  misc_feature (70)..(70): TAMRA-modified nucleotide

SEQ ID NO: 8 - DNA, 34 bp, Artificial Sequence
  Synthesized oligonucleotide
gtctcgtgggctcggagatgtgtataagagacag

SEQ ID NO: 9 - DNA, 19 bp, Artificial Sequence
  Synthesized oligonucleotide
  misc_feature (1)..(1): Phosphate-modified nucleotide
ctgtctcttatacacatct

SEQ ID NO: 10 - DNA, 58 bp, Artificial Sequence
  Synthesized oligonucleotide
  misc_feature (30)..(37): 8 bp index sequence
  misc_feature (30)..(37): n=a, t, g or c
aatgatacggcgaccaccgagatctacacnnnnnnnntcgtcggcagcgtcagatgtg

SEQ ID NO: 11 - DNA, 53 bp, Artificial Sequence
  Synthesized oligonucleotide
  misc_feature (25)..(32): 8 bp index sequence
  misc_feature (25)..(32): n=a, t, g or c
caagcagaagacggcatacgagatnnnnnnnngtctcgtgggctcggagatgt